European Patent Application EP 4 527 396 A1, published March 26, 2025. Title: THERAPEUTIC USE OF A POSTBIOTIC COMPOSITION FOR PSYCHIATRIC DISORDERS. Applicant: IGEN BIOLAB GROUP AG. Application EP, filed September 22, 2023. The sequence listing filed with the application follows.

SEQUENCE LISTING (8 sequences)

SEQ ID NO: 1 - DNA, 20 bp, Danio rerio
  source 1..20: mol_type = other DNA
  primer_bind 1..20
acctaccctcctcttggtcg

SEQ ID NO: 2 - DNA, 20 bp, Danio rerio
  source 1..20: mol_type = other DNA
  primer_bind 1..20
agaacacgccgcaacctttg

SEQ ID NO: 3 - DNA, 20 bp, Danio rerio
  source 1..20: mol_type = other DNA
  primer_bind 1..20
cgcagatcatccgggattca

SEQ ID NO: 4 - DNA, 20 bp, Danio rerio
  source 1..20: mol_type = other DNA
  primer_bind 1..20
actcatggcaagatccgcaa

SEQ ID NO: 5 - DNA, 20 bp, Danio rerio
  source 1..20: mol_type = other DNA
  primer_bind 1..20
tgtgtaagtgcatccggcag

SEQ ID NO: 6 - DNA, 20 bp, Danio rerio
  source 1..20: mol_type = other DNA
  primer_bind 1..20
atcagcaacaccaggtacgg

SEQ ID NO: 7 - DNA, 20 bp, Danio rerio
  source 1..20: mol_type = other DNA
  primer_bind 1..20
ctactcaactttcggggcgt

SEQ ID NO: 8 - DNA, 20 bp, Danio rerio
  source 1..20: mol_type = other DNA
  primer_bind 1..20
caccgccaagcatttatccg